European Patent Application EP 4 520 346 A1, published March 12, 2025. Title: CELLS, METHODS AND SYSTEM FOR USE IN THE TREATMENT OF A CANCER WITH DUAL-CAR-T. Applicant: Gyncentrum. Application EP. The sequence listing filed with the application follows.

SEQUENCE LISTING (38 sequences)

SEQ ID NO: 1 - DNA, 9652 bp, synthetic construct
  source 1..9652: mol_type = other DNA
acgcgtgtagtcttatgcaatactcttgtagtcttgcaacatggtaacgatgagttagcaacatgccttacaaggagagaaaaagcaccgtgcatgccgattggtggaagtaaggtggtacgatcgtgccttattaggaaggcaacagacgggtctgacatggattggacgaaccactgaattgccgcattgcagagatattgtatttaagtgcctagctcgatacaataaacgggtctctctggttagaccagatctgagcctgggagctctctggctaactagggaacccactgcttaagcctcaataaagcttgccttgagtgcttcaagtagtgtgtgcccgtctgttgtgtgactctggtaactagagatccctcagacccttttagtcagtgtggaaaatctctagcagtggcgcccgaacagggacttgaaagcgaaagggaaaccagaggagctctctcgacgcaggactcggcttgctgaagcgcgcacggcaagaggcgaggggcggcgactggtgagtacgccaaaaattttgactagcggaggctagaaggagagagatgggtgcgagagcgtcagtattaagcgggggagaattagatcgcgatgggaaaaaattcggttaaggccagggggaaagaaaaaatataaattaaaacatatagtatgggcaagcagggagctagaacgattcgcagttaatcctggcctgttagaaacatcagaaggctgtagacaaatactgggacagctacaaccatcccttcagacaggatcagaagaacttagatcattatataatacagtagcaaccctctattgtgtgcatcaaaggatagagataaaagacaccaaggaagctttagacaagatagaggaagagcaaaacaaaagtaagaccaccgcacagcaagcggccactgatcttcagacctggaggaggagatatgagggacaattggagaagtgaattatataaatataaagtagtaaaaattgaaccattaggagtagcacccaccaaggcaaagagaagagtggtgcagagagaaaaaagagcagtgggaataggagctttgttccttgggttcttgggagcagcaggaagcactatgggcgcagcgtcaatgacgctgacggtacaggccagacaattattgtctggtatagtgcagcagcagaacaatttgctgagggctattgaggcgcaacagcatctgttgcaactcacagtctggggcatcaagcagctccaggcaagaatcctggctgtggaaagatacctaaaggatcaacagctcctggggatttggggttgctctggaaaactcatttgcaccactgctgtgccttggaatgctagttggagtaataaatctctggaacagatttggaatcacacgacctggatggagtgggacagagaaattaacaattacacaagcttaatacactccttaattgaagaatcgcaaaaccagcaagaaaagaatgaacaagaattattggaattagataaatgggcaagtttgtggaattggtttaacataacaaattggctgtggtatataaaattattcataatgatagtaggaggcttggtaggtttaagaatagtttttgctgtactttctatagtgaatagagttaggcagggatattcaccattatcgtttcagacccacctcccaaccccgaggggacccgacaggcccgaaggaatagaagaagaaggtggagagagagacagagacagatccattcgattagtgaacggatctcgacggtatcggttaacttttaaaagaaaaggggggattggggggtacagtgcaggggaaagaatagtagacataatagcaacagacatacaaactaaagaattacaaaaacaaattacaaaattcaaaattttatcgatactagtattatgcccagtacatgaccttatgggactttcctacttggcagtacatctacgtattagtcatcgctattaccatggagtaattcatacaaaaggactcgcccctgccttggggaatcccagggaccgtcgttaaactcccactaacgtagaacccagagatcgctgcgttcccgccccctcacccgcccgctctcgtcatcactgaggtggagaagagcatgcgtgaggctccggtgcccgtcagtgggcagagcgcacatcgcccacagtccccgagaagttggggggaggggtcggcaattgaaccggtgcctagagaaggtggcgcggggtaaactgggaaagtgatgtcgtgtactggctccgcctttttcccgagggtgggggagaaccgtatataagtgcagtagtcgccgtgaacgttctttttcgcaacgggtttgccgccagaacacaggtaagtgccgtgtgtggttcccgcgggcctggcctctttacgggttatggcccttgcgtgccttgaattacttccacgcccctggctgcagtacgtgattcttgatcccgagcttcgggttggaagtgggtgggagagttcgaggccttgcgcttaaggagccccttcgcctcgtgcttgagttgaggcctggcttgggcgctggggccgccgcgtgcgaatctggtggcaccttcgcgcctgtctcgctgctttcgataagtctctagccatttaaaatttttgatgacctgctgcgacgctttttttctggcaagatagtcttgtaaatgcgggccaagatctgcacactggtatttcggtttttggggccgcgggcggcgacggggcccgtgcgtcccagcgcacatgttcggcgaggcggggcctgcgagcgcggccaccgagaatcggacgggggtagtctcaagctggccggcctgctctggtgcctggcctcgcgccgccgtgtatcgccccgccctgggcggcaaggctggcccggtcggcaccagttgcgtgagcggaaagatggccgcttcccggccctgctgcagggagctcaaaatggaggacgcggcgctcgggagagcgggcgggtgagtcacccacacaaaggaaaagggcctttccgtcctcagccgtcgcttcatgtgactccacggagtaccgggcgccgtccaggcacctcgattagttctcgagcttttggagtacgtcgtctttaggttggggggaggggttttatgcgatggagtttccccacactgagtgggtggagactgaagttaggccagcttggcacttgatgtaattctccttggaatttgccctttttgagtttggatcttggttcattctcaagcctcagacagtggttcaaagtttttttcttccatttcaggtgtcgtgattcgaagccgccaccatggccttaccagtgaccgccttgctcctgccgctggccttgctgctccacgccgccaggccgagctccgagctgacccaggatcccgccgtgagcgtggccctgggacagacagtgaggatcacctgtcagggcgactccctgagatcctactacgcctcctggtaccagcagaagcccggccaggcccccgtgctggttatctacggcaagaataataggcctagcggcatccctgatagattttccggcagctccagcggcaataccgccagcctgaccatcaccggcgcccaggctgaggacgaggccgattactactgcaattccagggacagcagcggcaatcctcctgtggtgtttggcggcggcaccaagctgacagtgctgggcagcaggggcggcggaggatctggaggaggcggatccggcggcggaggttctctggagatggcccaggtgcagctggtggagagcggcggaggcctggtgcacccaggaggatccctgagactgagctgtgccgcctccggcttcacctttaggtcccacagcatgaattgggtgagacaggcccctggcaagggcctggagtgggtgtccagcatcagcagcgacagcacctacacctactacgccgatagcgtgaagggcaggttcaccatctccagagacaacgccaagaatagcctgtacctgcagatgaacagcctgagggccgaggataccgccgtgtactactgcgccagaagcggcggccagtggaagtactacgactactggggccagggcacactggtgacagtgagctccaccactaccccagcaccgaggccacccaccccggctcctaccatcgcctcccagcctctgtccctgcgtccggaggcatgtagacccgcagctggtggggccgtgcatacccggggtcttgacttcgcctgcgatttctggctgcccatcggctgcgccgccttcgtggtggtgtgtatcctgggctgtatcctgatctgttggctgacaaagaagaagtactccagctccgtgcacgatcccaatggcgagtacatgtttatgagagccgtgaataccgccaagaagagcagactgaccgacgtgaccctgaagcgcggtcggaagaagctgctgtacatctttaagcaacccttcatgaggcctgtgcagactactcaagaggaggacggctgttcatgccggttcccagaggaggaggaaggcggctgcgaactgcgcgtgaaattcagccgcagcgcagatgctccagcctacaagcaggggcagaaccagctctacaacgaactcaatcttggtcggagagaggagtacgacgtgctggacaagcggagaggacgggacccagaaatgggcgggaagccgcgcagaaagaatccccaagagggcctgtacaacgagctccaaaaggataagatggcagaagcctatagcgagattggtatgaaaggggaacgcagaagaggcaaaggccacgacggactgtaccagggactcagcaccgccaccaaggacacctatgacgctcttcacatgcaggccctgccgcctcgggagggcagaggcagcctgctgacatgtggcgacgtggaagagaaccctggccccatggtgagcaagggcgaggagctgttcaccggggtggtgcccatcctggtcgagctggacggcgacgtaaacggccacaagttcagcgtgtccggcgagggcgagggcgatgccacctacggcaagctgaccctgaagttcatctgcaccaccggcaagctgcccgtgccctggcccaccctcgtgaccaccctgacctacggcgtgcagtgcttcagccgctaccccgaccacatgaagcagcacgacttcttcaagtccgccatgcccgaaggctacgtccaggagcgcaccatcttcttcaaggacgacggcaactacaagacccgcgccgaggtgaagttcgagggcgacaccctggtgaaccgcatcgagctgaagggcatcgacttcaaggaggacggcaacatcctggggcacaagctggagtacaactacaacagccacaacgtctatatcatggccgacaagcagaagaacggcatcaaggtgaacttcaagatccgccacaacatcgaggacggcagcgtgcagctcgccgaccactaccagcagaacacccccatcggcgacggccccgtgctgctgcccgacaaccactacctgagcacccagtccgccctgagcaaagaccccaacgagaagcgcgatcacatggtcctgctggagttcgtgaccgccgccgggatcactctcggcatggacgagctgtacaagtaatctagaaatcaacctctggattacaaaatttgtgaaagattgactggtattcttaactatgttgctccttttacgctatgtggatacgctgctttaatgcctttgtatcatgctattgcttcccgtatggctttcattttctcctccttgtataaatcctggttgctgtctctttatgaggagttgtggcccgttgtcaggcaacgtggcgtggtgtgcactgtgtttgctgacgcaacccccactggttggggcattgccaccacctgtcagctcctttccgggactttcgctttccccctccctattgccacggcggaactcatcgccgcctgccttgcccgctgctggacaggggctcggctgttgggcactgacaattccgtggtgttgtcggggaaatcatcgtcctttccttggctgctcgcctgtgttgccacctggattctgcgcgggacgtccttctgctacgtcccttcggccctcaatccagcggaccttccttcccgcggcctgctgccggctctgcggcctcttccgcgtcttcgccttcgccctcagacgagtcggatctccctttgggccgcctccccgcctggtacctttaagaccaatgacttacaaggcagctgtagatcttagccactttttaaaagaaaaggggggactggaagggctaattcactcccaacgaagataagatctgctttttgcttgtactgggtctctctggttagaccagatctgagcctgggagctctctggctaactagggaacccactgcttaagcctcaataaagcttgccttgagtgcttcaagtagtgtgtgcccgtctgttgtgtgactctggtaactagagatccctcagacccttttagtcagtgtggaaaatctctagcagtagtagttcatgtcatcttattattcagtatttataacttgcaaagaaatgaatatcagagagtgagaggaacttgtttattgcagcttataatggttacaaataaagcaatagcatcacaaatttcacaaataaagcatttttttcactgcattctagttgtggtttgtccaaactcatcaatgtatcttatcatgtctggctctagctatcccgcccctaactccgcccatcccgcccctaactccgcccagttccgcccattctccgccccatggctgactaattttttttatttatgcagaggccgaggccgcctcggcctctgagctattccagaagtagtgaggaggcttttttggaggcctagacttttgcagagaccaaattcgtaatcatgtcatagctgtttcctgtgtgaaattgttatccgctcacaattccacacaacatacgagccggaagcataaagtgtaaagcctggggtgcctaatgagtgagctaactcacattaattgcgttgcgctcactgcccgctttccagtcgggaaacctgtcgtgccagctgcattaatgaatcggccaacgcgcggggagaggcggtttgcgtattgggcgctcttccgcttcctcgctcactgactcgctgcgctcggtcgttcggctgcggcgagcggtatcagctcactcaaaggcggtaatacggttatccacagaatcaggggataacgcaggaaagaacatgtgagcaaaaggccagcaaaaggccaggaaccgtaaaaaggccgcgttgctggcgtttttccataggctccgcccccctgacgagcatcacaaaaatcgacgctcaagtcagaggtggcgaaacccgacaggactataaagataccaggcgtttccccctggaagctccctcgtgcgctctcctgttccgaccctgccgcttaccggatacctgtccgcctttctcccttcgggaagcgtggcgctttctcatagctcacgctgtaggtatctcagttcggtgtaggtcgttcgctccaagctgggctgtgtgcacgaaccccccgttcagcccgaccgctgcgccttatccggtaactatcgtcttgagtccaacccggtaagacacgacttatcgccactggcagcagccactggtaacaggattagcagagcgaggtatgtaggcggtgctacagagttcttgaagtggtggcctaactacggctacactagaagaacagtatttggtatctgcgctctgctgaagccagttaccttcggaaaaagagttggtagctcttgatccggcaaacaaaccaccgctggtagcggtggtttttttgtttgcaagcagcagattacgcgcagaaaaaaaggatctcaagaagatcctttgatcttttctacggggtctgacgctcagtggaacgaaaactcacgttaagggattttggtcatgagattatcaaaaaggatcttcacctagatccttttaaattaaaaatgaagttttaaatcaatctaaagtatatatgagtaaacttggtctgacagttaccaatgcttaatcagtgaggcacctatctcagcgatctgtctatttcgttcatccatagttgcctgactccccgtcgtgtagataactacgatacgggagggcttaccatctggccccagtgctgcaatgataccgcgagacccacgctcaccggctccagatttatcagcaataaaccagccagccggaagggccgagcgcagaagtggtcctgcaactttatccgcctccatccagtctattaattgttgccgggaagctagagtaagtagttcgccagttaatagtttgcgcaacgttgttgccattgctacaggcatcgtggtgtcacgctcgtcgtttggtatggcttcattcagctccggttcccaacgatcaaggcgagttacatgatcccccatgttgtgcaaaaaagcggttagctccttcggtcctccgatcgttgtcagaagtaagttggccgcagtgttatcactcatggttatggcagcactgcataattctcttactgtcatgccatccgtaagatgcttttctgtgactggtgagtactcaaccaagtcattctgagaatagtgtatgcggcgaccgagttgctcttgcccggcgtcaatacgggataataccgcgccacatagcagaactttaaaagtgctcatcattggaaaacgttcttcggggcgaaaactctcaaggatcttaccgctgttgagatccagttcgatgtaacccactcgtgcacccaactgatcttcagcatcttttactttcaccagcgtttctgggtgagcaaaaacaggaaggcaaaatgccgcaaaaaagggaataagggcgacacggaaatgttgaatactcatactcttcctttttcaatattattgaagcatttatcagggttattgtctcatgagcggatacatatttgaatgtatttagaaaaataaacaaataggggttccgcgcacatttccccgaaaagtgccacctgacgtctaagaaaccattattatcatgacattaacctataaaaataggcgtatcacgaggccctttcgtctcgcgcgtttcggtgatgacggtgaaaacctctgacacatgcagctcccggagacggtcacagcttgtctgtaagcggatgccgggagcagacaagcccgtcagggcgcgtcagcgggtgttggcgggtgtcggggctggcttaactatgcggcatcagagcagattgtactgagagtgcaccatatgcggtgtgaaataccgcacagatgcgtaaggagaaaataccgcatcaggcgccattcgccattcaggctgcgcaactgttgggaagggcgatcggtgcgggcctcttcgctattacgccagctggcgaaagggggatgtgctgcaaggcgattaagttgggtaacgccagggttttcccagtcacgacgttgtaaaacgacggccagtgccaagctg

SEQ ID NO: 2 - DNA, 1656 bp, synthetic construct
  source 1..1656: mol_type = other DNA
ttcgaagccgccaccatggccttaccagtgaccgccttgctcctgccgctggccttgctgctccacgccgccaggccgagctccgagctgacccaggatcccgccgtgagcgtggccctgggacagacagtgaggatcacctgtcagggcgactccctgagatcctactacgcctcctggtaccagcagaagcccggccaggcccccgtgctggttatctacggcaagaataataggcctagcggcatccctgatagattttccggcagctccagcggcaataccgccagcctgaccatcaccggcgcccaggctgaggacgaggccgattactactgcaattccagggacagcagcggcaatcctcctgtggtgtttggcggcggcaccaagctgacagtgctgggcagcaggggcggcggaggatctggaggaggcggatccggcggcggaggttctctggagatggcccaggtgcagctggtggagagcggcggaggcctggtgcacccaggaggatccctgagactgagctgtgccgcctccggcttcacctttaggtcccacagcatgaattgggtgagacaggcccctggcaagggcctggagtgggtgtccagcatcagcagcgacagcacctacacctactacgccgatagcgtgaagggcaggttcaccatctccagagacaacgccaagaatagcctgtacctgcagatgaacagcctgagggccgaggataccgccgtgtactactgcgccagaagcggcggccagtggaagtactacgactactggggccagggcacactggtgacagtgagctccaccactaccccagcaccgaggccacccaccccggctcctaccatcgcctcccagcctctgtccctgcgtccggaggcatgtagacccgcagctggtggggccgtgcatacccggggtcttgacttcgcctgcgatttctggctgcccatcggctgcgccgccttcgtggtggtgtgtatcctgggctgtatcctgatctgttggctgacaaagaagaagtactccagctccgtgcacgatcccaatggcgagtacatgtttatgagagccgtgaataccgccaagaagagcagactgaccgacgtgaccctgaagcgcggtcggaagaagctgctgtacatctttaagcaacccttcatgaggcctgtgcagactactcaagaggaggacggctgttcatgccggttcccagaggaggaggaaggcggctgcgaactgcgcgtgaaattcagccgcagcgcagatgctccagcctacaagcaggggcagaaccagctctacaacgaactcaatcttggtcggagagaggagtacgacgtgctggacaagcggagaggacgggacccagaaatgggcgggaagccgcgcagaaagaatccccaagagggcctgtacaacgagctccaaaaggataagatggcagaagcctatagcgagattggtatgaaaggggaacgcagaagaggcaaaggccacgacggactgtaccagggactcagcaccgccaccaaggacacctatgacgctcttcacatgcaggccctgccgcctcgggagggcagaggcagcctgctgacatgtggcgacgtggaagagaaccctggcccc

SEQ ID NO: 3 - DNA, 9634 bp, synthetic construct
  source 1..9634: mol_type = other DNA
acgcgtgtagtcttatgcaatactcttgtagtcttgcaacatggtaacgatgagttagcaacatgccttacaaggagagaaaaagcaccgtgcatgccgattggtggaagtaaggtggtacgatcgtgccttattaggaaggcaacagacgggtctgacatggattggacgaaccactgaattgccgcattgcagagatattgtatttaagtgcctagctcgatacaataaacgggtctctctggttagaccagatctgagcctgggagctctctggctaactagggaacccactgcttaagcctcaataaagcttgccttgagtgcttcaagtagtgtgtgcccgtctgttgtgtgactctggtaactagagatccctcagacccttttagtcagtgtggaaaatctctagcagtggcgcccgaacagggacttgaaagcgaaagggaaaccagaggagctctctcgacgcaggactcggcttgctgaagcgcgcacggcaagaggcgaggggcggcgactggtgagtacgccaaaaattttgactagcggaggctagaaggagagagatgggtgcgagagcgtcagtattaagcgggggagaattagatcgcgatgggaaaaaattcggttaaggccagggggaaagaaaaaatataaattaaaacatatagtatgggcaagcagggagctagaacgattcgcagttaatcctggcctgttagaaacatcagaaggctgtagacaaatactgggacagctacaaccatcccttcagacaggatcagaagaacttagatcattatataatacagtagcaaccctctattgtgtgcatcaaaggatagagataaaagacaccaaggaagctttagacaagatagaggaagagcaaaacaaaagtaagaccaccgcacagcaagcggccactgatcttcagacctggaggaggagatatgagggacaattggagaagtgaattatataaatataaagtagtaaaaattgaaccattaggagtagcacccaccaaggcaaagagaagagtggtgcagagagaaaaaagagcagtgggaataggagctttgttccttgggttcttgggagcagcaggaagcactatgggcgcagcgtcaatgacgctgacggtacaggccagacaattattgtctggtatagtgcagcagcagaacaatttgctgagggctattgaggcgcaacagcatctgttgcaactcacagtctggggcatcaagcagctccaggcaagaatcctggctgtggaaagatacctaaaggatcaacagctcctggggatttggggttgctctggaaaactcatttgcaccactgctgtgccttggaatgctagttggagtaataaatctctggaacagatttggaatcacacgacctggatggagtgggacagagaaattaacaattacacaagcttaatacactccttaattgaagaatcgcaaaaccagcaagaaaagaatgaacaagaattattggaattagataaatgggcaagtttgtggaattggtttaacataacaaattggctgtggtatataaaattattcataatgatagtaggaggcttggtaggtttaagaatagtttttgctgtactttctatagtgaatagagttaggcagggatattcaccattatcgtttcagacccacctcccaaccccgaggggacccgacaggcccgaaggaatagaagaagaaggtggagagagagacagagacagatccattcgattagtgaacggatctcgacggtatcggttaacttttaaaagaaaaggggggattggggggtacagtgcaggggaaagaatagtagacataatagcaacagacatacaaactaaagaattacaaaaacaaattacaaaattcaaaattttatcgatactagtattatgcccagtacatgaccttatgggactttcctacttggcagtacatctacgtattagtcatcgctattaccatggagtaattcatacaaaaggactcgcccctgccttggggaatcccagggaccgtcgttaaactcccactaacgtagaacccagagatcgctgcgttcccgccccctcacccgcccgctctcgtcatcactgaggtggagaagagcatgcgtgaggctccggtgcccgtcagtgggcagagcgcacatcgcccacagtccccgagaagttggggggaggggtcggcaattgaaccggtgcctagagaaggtggcgcggggtaaactgggaaagtgatgtcgtgtactggctccgcctttttcccgagggtgggggagaaccgtatataagtgcagtagtcgccgtgaacgttctttttcgcaacgggtttgccgccagaacacaggtaagtgccgtgtgtggttcccgcgggcctggcctctttacgggttatggcccttgcgtgccttgaattacttccacgcccctggctgcagtacgtgattcttgatcccgagcttcgggttggaagtgggtgggagagttcgaggccttgcgcttaaggagccccttcgcctcgtgcttgagttgaggcctggcttgggcgctggggccgccgcgtgcgaatctggtggcaccttcgcgcctgtctcgctgctttcgataagtctctagccatttaaaatttttgatgacctgctgcgacgctttttttctggcaagatagtcttgtaaatgcgggccaagatctgcacactggtatttcggtttttggggccgcgggcggcgacggggcccgtgcgtcccagcgcacatgttcggcgaggcggggcctgcgagcgcggccaccgagaatcggacgggggtagtctcaagctggccggcctgctctggtgcctggcctcgcgccgccgtgtatcgccccgccctgggcggcaaggctggcccggtcggcaccagttgcgtgagcggaaagatggccgcttcccggccctgctgcagggagctcaaaatggaggacgcggcgctcgggagagcgggcgggtgagtcacccacacaaaggaaaagggcctttccgtcctcagccgtcgcttcatgtgactccacggagtaccgggcgccgtccaggcacctcgattagttctcgagcttttggagtacgtcgtctttaggttggggggaggggttttatgcgatggagtttccccacactgagtgggtggagactgaagttaggccagcttggcacttgatgtaattctccttggaatttgccctttttgagtttggatcttggttcattctcaagcctcagacagtggttcaaagtttttttcttccatttcaggtgtcgtgattcgaagccgccaccatggccttaccagtgaccgccttgctcctgccgctggccttgctgctccacgccgccaggccggaggtgcagctgctggagtccggcggcggactggtgcagccaggaggatccctgaggctgtcctgcgccgccagcggattcactttcagatcctacgccatgagctgggtgagacaggcccctggcaagggcctggagtgggtgtccgccatctccggcggcggtggaaatacattctacgccgactccgtgaagggcaggttcacaatcagcagggacaattccaagaacaccctgtacctgcagatgaactccctgagggccgaggacaccgccgtgtactactgcgccaaggtgaggcccttttggggcacctttgattactggggccagggcaccctggtgacagtgtccagcggcggcggcggaagcggaggaggaggatctggcggcggcggtagcgagatcgtgctgacccagtcccccggcacactgtccctgtcccccggagagagagccaccctgtcctgcagggcctcccagtccgtgagctccagctacctggcctggtaccagcagaagcccggccaggcccccaggctgctgatctacggcgcctcctccagagccacaggcatccctgacaggttcagcggcagcggctccggcacagactttacactgacaatctccagactggagcctgaggatttcgccgtgtactattgtcagcagtacttcaaccctcctgagtacacattcggccagggcacaaaggtggagatcaagagaaccactaccccagcaccgaggccacccaccccggctcctaccatcgcctcccagcctctgtccctgcgtccggaggcatgtagacccgcagctggtggggccgtgcatacccggggtcttgacttcgcctgcgatatctacatttgggcccctctggctggtacttgcggggtcctgctgctttcactcgtgatcactctttactgtaggagcaagcggagcagactgctgcacagcgactacatgaacatgaccccccggaggcctggccccacccggaagcactaccagccctacgcccctcccagggatttcgccgcctaccggagcagagaccagagactgccccctgacgcccacaagccccccggaggaggaagctttagaacacccatccaggaggagcaggccgacgcccacagcacactggccaagatccgcgtgaaattcagccgcagcgcagatgctccagcctacaagcaggggcagaaccagctctacaacgaactcaatcttggtcggagagaggagtacgacgtgctggacaagcggagaggacgggacccagaaatgggcgggaagccgcgcagaaagaatccccaagagggcctgtacaacgagctccaaaaggataagatggcagaagcctatagcgagattggtatgaaaggggaacgcagaagaggcaaaggccacgacggactgtaccagggactcagcaccgccaccaaggacacctatgacgctcttcacatgcaggccctgccgcctcgggagggcagaggcagcctgctgacatgtggcgacgtggaagagaaccctggccccatggtgagcaagggcgaggagctgttcaccggggtggtgcccatcctggtcgagctggacggcgacgtaaacggccacaagttcagcgtgtccggcgagggcgagggcgatgccacctacggcaagctgaccctgaagttcatctgcaccaccggcaagctgcccgtgccctggcccaccctcgtgaccaccctgacctacggcgtgcagtgcttcagccgctaccccgaccacatgaagcagcacgacttcttcaagtccgccatgcccgaaggctacgtccaggagcgcaccatcttcttcaaggacgacggcaactacaagacccgcgccgaggtgaagttcgagggcgacaccctggtgaaccgcatcgagctgaagggcatcgacttcaaggaggacggcaacatcctggggcacaagctggagtacaactacaacagccacaacgtctatatcatggccgacaagcagaagaacggcatcaaggtgaacttcaagatccgccacaacatcgaggacggcagcgtgcagctcgccgaccactaccagcagaacacccccatcggcgacggccccgtgctgctgcccgacaaccactacctgagcacccagtccgccctgagcaaagaccccaacgagaagcgcgatcacatggtcctgctggagttcgtgaccgccgccgggatcactctcggcatggacgagctgtacaagtaatctagaaatcaacctctggattacaaaatttgtgaaagattgactggtattcttaactatgttgctccttttacgctatgtggatacgctgctttaatgcctttgtatcatgctattgcttcccgtatggctttcattttctcctccttgtataaatcctggttgctgtctctttatgaggagttgtggcccgttgtcaggcaacgtggcgtggtgtgcactgtgtttgctgacgcaacccccactggttggggcattgccaccacctgtcagctcctttccgggactttcgctttccccctccctattgccacggcggaactcatcgccgcctgccttgcccgctgctggacaggggctcggctgttgggcactgacaattccgtggtgttgtcggggaaatcatcgtcctttccttggctgctcgcctgtgttgccacctggattctgcgcgggacgtccttctgctacgtcccttcggccctcaatccagcggaccttccttcccgcggcctgctgccggctctgcggcctcttccgcgtcttcgccttcgccctcagacgagtcggatctccctttgggccgcctccccgcctggtacctttaagaccaatgacttacaaggcagctgtagatcttagccactttttaaaagaaaaggggggactggaagggctaattcactcccaacgaagataagatctgctttttgcttgtactgggtctctctggttagaccagatctgagcctgggagctctctggctaactagggaacccactgcttaagcctcaataaagcttgccttgagtgcttcaagtagtgtgtgcccgtctgttgtgtgactctggtaactagagatccctcagacccttttagtcagtgtggaaaatctctagcagtagtagttcatgtcatcttattattcagtatttataacttgcaaagaaatgaatatcagagagtgagaggaacttgtttattgcagcttataatggttacaaataaagcaatagcatcacaaatttcacaaataaagcatttttttcactgcattctagttgtggtttgtccaaactcatcaatgtatcttatcatgtctggctctagctatcccgcccctaactccgcccatcccgcccctaactccgcccagttccgcccattctccgccccatggctgactaattttttttatttatgcagaggccgaggccgcctcggcctctgagctattccagaagtagtgaggaggcttttttggaggcctagacttttgcagagaccaaattcgtaatcatgtcatagctgtttcctgtgtgaaattgttatccgctcacaattccacacaacatacgagccggaagcataaagtgtaaagcctggggtgcctaatgagtgagctaactcacattaattgcgttgcgctcactgcccgctttccagtcgggaaacctgtcgtgccagctgcattaatgaatcggccaacgcgcggggagaggcggtttgcgtattgggcgctcttccgcttcctcgctcactgactcgctgcgctcggtcgttcggctgcggcgagcggtatcagctcactcaaaggcggtaatacggttatccacagaatcaggggataacgcaggaaagaacatgtgagcaaaaggccagcaaaaggccaggaaccgtaaaaaggccgcgttgctggcgtttttccataggctccgcccccctgacgagcatcacaaaaatcgacgctcaagtcagaggtggcgaaacccgacaggactataaagataccaggcgtttccccctggaagctccctcgtgcgctctcctgttccgaccctgccgcttaccggatacctgtccgcctttctcccttcgggaagcgtggcgctttctcatagctcacgctgtaggtatctcagttcggtgtaggtcgttcgctccaagctgggctgtgtgcacgaaccccccgttcagcccgaccgctgcgccttatccggtaactatcgtcttgagtccaacccggtaagacacgacttatcgccactggcagcagccactggtaacaggattagcagagcgaggtatgtaggcggtgctacagagttcttgaagtggtggcctaactacggctacactagaagaacagtatttggtatctgcgctctgctgaagccagttaccttcggaaaaagagttggtagctcttgatccggcaaacaaaccaccgctggtagcggtggtttttttgtttgcaagcagcagattacgcgcagaaaaaaaggatctcaagaagatcctttgatcttttctacggggtctgacgctcagtggaacgaaaactcacgttaagggattttggtcatgagattatcaaaaaggatcttcacctagatccttttaaattaaaaatgaagttttaaatcaatctaaagtatatatgagtaaacttggtctgacagttaccaatgcttaatcagtgaggcacctatctcagcgatctgtctatttcgttcatccatagttgcctgactccccgtcgtgtagataactacgatacgggagggcttaccatctggccccagtgctgcaatgataccgcgagacccacgctcaccggctccagatttatcagcaataaaccagccagccggaagggccgagcgcagaagtggtcctgcaactttatccgcctccatccagtctattaattgttgccgggaagctagagtaagtagttcgccagttaatagtttgcgcaacgttgttgccattgctacaggcatcgtggtgtcacgctcgtcgtttggtatggcttcattcagctccggttcccaacgatcaaggcgagttacatgatcccccatgttgtgcaaaaaagcggttagctccttcggtcctccgatcgttgtcagaagtaagttggccgcagtgttatcactcatggttatggcagcactgcataattctcttactgtcatgccatccgtaagatgcttttctgtgactggtgagtactcaaccaagtcattctgagaatagtgtatgcggcgaccgagttgctcttgcccggcgtcaatacgggataataccgcgccacatagcagaactttaaaagtgctcatcattggaaaacgttcttcggggcgaaaactctcaaggatcttaccgctgttgagatccagttcgatgtaacccactcgtgcacccaactgatcttcagcatcttttactttcaccagcgtttctgggtgagcaaaaacaggaaggcaaaatgccgcaaaaaagggaataagggcgacacggaaatgttgaatactcatactcttcctttttcaatattattgaagcatttatcagggttattgtctcatgagcggatacatatttgaatgtatttagaaaaataaacaaataggggttccgcgcacatttccccgaaaagtgccacctgacgtctaagaaaccattattatcatgacattaacctataaaaataggcgtatcacgaggccctttcgtctcgcgcgtttcggtgatgacggtgaaaacctctgacacatgcagctcccggagacggtcacagcttgtctgtaagcggatgccgggagcagacaagcccgtcagggcgcgtcagcgggtgttggcgggtgtcggggctggcttaactatgcggcatcagagcagattgtactgagagtgcaccatatgcggtgtgaaataccgcacagatgcgtaaggagaaaataccgcatcaggcgccattcgccattcaggctgcgcaactgttgggaagggcgatcggtgcgggcctcttcgctattacgccagctggcgaaagggggatgtgctgcaaggcgattaagttgggtaacgccagggttttcccagtcacgacgttgtaaaacgacggccagtgccaagctg

SEQ ID NO: 4 - DNA, 1638 bp, synthetic construct
  source 1..1638: mol_type = other DNA
ttcgaagccgccaccatggccttaccagtgaccgccttgctcctgccgctggccttgctgctccacgccgccaggccggaggtgcagctgctggagtccggcggcggactggtgcagccaggaggatccctgaggctgtcctgcgccgccagcggattcactttcagatcctacgccatgagctgggtgagacaggcccctggcaagggcctggagtgggtgtccgccatctccggcggcggtggaaatacattctacgccgactccgtgaagggcaggttcacaatcagcagggacaattccaagaacaccctgtacctgcagatgaactccctgagggccgaggacaccgccgtgtactactgcgccaaggtgaggcccttttggggcacctttgattactggggccagggcaccctggtgacagtgtccagcggcggcggcggaagcggaggaggaggatctggcggcggcggtagcgagatcgtgctgacccagtcccccggcacactgtccctgtcccccggagagagagccaccctgtcctgcagggcctcccagtccgtgagctccagctacctggcctggtaccagcagaagcccggccaggcccccaggctgctgatctacggcgcctcctccagagccacaggcatccctgacaggttcagcggcagcggctccggcacagactttacactgacaatctccagactggagcctgaggatttcgccgtgtactattgtcagcagtacttcaaccctcctgagtacacattcggccagggcacaaaggtggagatcaagagaaccactaccccagcaccgaggccacccaccccggctcctaccatcgcctcccagcctctgtccctgcgtccggaggcatgtagacccgcagctggtggggccgtgcatacccggggtcttgacttcgcctgcgatatctacatttgggcccctctggctggtacttgcggggtcctgctgctttcactcgtgatcactctttactgtaggagcaagcggagcagactgctgcacagcgactacatgaacatgaccccccggaggcctggccccacccggaagcactaccagccctacgcccctcccagggatttcgccgcctaccggagcagagaccagagactgccccctgacgcccacaagccccccggaggaggaagctttagaacacccatccaggaggagcaggccgacgcccacagcacactggccaagatccgcgtgaaattcagccgcagcgcagatgctccagcctacaagcaggggcagaaccagctctacaacgaactcaatcttggtcggagagaggagtacgacgtgctggacaagcggagaggacgggacccagaaatgggcgggaagccgcgcagaaagaatccccaagagggcctgtacaacgagctccaaaaggataagatggcagaagcctatagcgagattggtatgaaaggggaacgcagaagaggcaaaggccacgacggactgtaccagggactcagcaccgccaccaaggacacctatgacgctcttcacatgcaggccctgccgcctcgggagggcagaggcagcctgctgacatgtggcgacgtggaagagaaccctggcccc

SEQ ID NO: 5 - DNA, 20 bp, synthetic construct
  source 1..20: mol_type = other DNA
ggggaggggttttatgcgat

SEQ ID NO: 6 - DNA, 20 bp, synthetic construct
  source 1..20: mol_type = other DNA
gaatgtatttccaccgccgc

SEQ ID NO: 7 - DNA, 20 bp, synthetic construct
  source 1..20: mol_type = other DNA
ccccggaggaggaagcttta

SEQ ID NO: 8 - DNA, 20 bp, synthetic construct
  source 1..20: mol_type = other DNA
aggccctcttggggattctt

SEQ ID NO: 9 - DNA, 20 bp, synthetic construct
  source 1..20: mol_type = other DNA
cctgagtacacattcggcca

SEQ ID NO: 10 - DNA, 20 bp, synthetic construct
  source 1..20: mol_type = other DNA
cgtagggctggtagtgcttc

SEQ ID NO: 11 - DNA, 20 bp, synthetic construct
  source 1..20: mol_type = other DNA
catttctgggtcccgtcctc

SEQ ID NO: 12 - DNA, 20 bp, synthetic construct
  source 1..20: mol_type = other DNA
ctacatttgggcccctctgg

SEQ ID NO: 13 - DNA, 20 bp, synthetic construct
  source 1..20: mol_type = other DNA
gtactactgcgccaaggtga

SEQ ID NO: 14 - DNA, 20 bp, synthetic construct
  source 1..20: mol_type = other DNA
cagaggggcccaaatgtaga

SEQ ID NO: 15 - DNA, 20 bp, synthetic construct
  source 1..20: mol_type = other DNA
gccagcggattcactttcag

SEQ ID NO: 16 - DNA, 20 bp, synthetic construct
  source 1..20: mol_type = other DNA
gctgaacctgtcagggatgc

SEQ ID NO: 17 - DNA, 20 bp, synthetic construct
  source 1..20: mol_type = other DNA
atagcgtgaagggcaggttc

SEQ ID NO: 18 - DNA, 20 bp, synthetic construct
  source 1..20: mol_type = other DNA
tgtactcgccattgggatcg

SEQ ID NO: 19 - DNA, 20 bp, synthetic construct
  source 1..20: mol_type = other DNA
ccccgtgctggttatctacg

SEQ ID NO: 20 - DNA, 20 bp, synthetic construct
  source 1..20: mol_type = other DNA
aacctgcccttcacgctatc

SEQ ID NO: 21 - DNA, 20 bp, synthetic construct
  source 1..20: mol_type = other DNA
cactgagtgggtggagactg

SEQ ID NO: 22 - DNA, 20 bp, synthetic construct
  source 1..20: mol_type = other DNA
tgcagtagtaatcggcctcg

SEQ ID NO: 23 - DNA, 20 bp, synthetic construct
  source 1..20: mol_type = other DNA
ctgaggacgaggccgattac

SEQ ID NO: 24 - DNA, 20 bp, synthetic construct
  source 1..20: mol_type = other DNA
aatcgcaggcgaagtcaaga

SEQ ID NO: 25 - DNA, 20 bp, synthetic construct
  source 1..20: mol_type = other DNA
tcttgacttcgcctgcgatt

SEQ ID NO: 26 - DNA, 20 bp, synthetic construct
  source 1..20: mol_type = other DNA
catttctgggtcccgtcctc

SEQ ID NO: 27 - DNA, 20 bp, synthetic construct
  source 1..20: mol_type = other DNA
acattctacgccgactccgt

SEQ ID NO: 28 - DNA, 20 bp, synthetic construct
  source 1..20: mol_type = other DNA
cccagtaatcaaaggtgccc

SEQ ID NO: 29 - DNA, 18 bp, synthetic construct
  source 1..18: mol_type = other DNA
gcggcatccctgatagat

SEQ ID NO: 30 - DNA, 20 bp, synthetic construct
  source 1..20: mol_type = other DNA
caaacaccacaggaggattg

SEQ ID NO: 31 - DNA, 20 bp, synthetic construct
  source 1..20: mol_type = other DNA
caagcctcagacagtggttc

SEQ ID NO: 32 - DNA, 20 bp, synthetic construct
  source 1..20: mol_type = other DNA
caaggcggtcactggtaagg

SEQ ID NO: 33 - DNA, 20 bp, synthetic construct
  source 1..20: mol_type = other DNA
acattctacgccgactccgt

SEQ ID NO: 34 - DNA, 20 bp, synthetic construct
  source 1..20: mol_type = other DNA
cccagtaatcaaaggtgccc

SEQ ID NO: 35 - DNA, 18 bp, synthetic construct
  source 1..18: mol_type = other DNA
gcggcatccctgatagat

SEQ ID NO: 36 - DNA, 20 bp, synthetic construct
  source 1..20: mol_type = other DNA
caaacaccacaggaggattg

SEQ ID NO: 37 - DNA, 25 bp, synthetic construct
  source 1..25: mol_type = other DNA
ttgtccctgctgattgtgaacctgc

SEQ ID NO: 38 - DNA, 26 bp, synthetic construct
  source 1..26: mol_type = other DNA
acgaggccgattactactgcaattcc